European Patent Application EP 4 509 594 A1, published February 19, 2025. Title: 신규한 미생물 및 이를 포함하는 조성물. Applicant: 서울대학교 산학협력단. Application KR. The sequence listing filed with the application follows.

SEQUENCE LISTING (30 sequences)

SEQ ID NO: 1 - DNA, 24 bp, synthetic construct
  source 1..24: mol_type = other DNA
acccgaaactgatgctgtggatag

SEQ ID NO: 2 - DNA, 24 bp, synthetic construct
  source 1..24: mol_type = other DNA
aaatggccgggcagaacttgtgta

SEQ ID NO: 3 - DNA, 19 bp, synthetic construct
  source 1..19: mol_type = other DNA
atgtccggccgatgctctc

SEQ ID NO: 4 - DNA, 23 bp, synthetic construct
  source 1..23: mol_type = other DNA
tttggctgctcttgggtctgtat

SEQ ID NO: 5 - DNA, 23 bp, synthetic construct
  source 1..23: mol_type = other DNA
caccctgacatagacagtgaaag

SEQ ID NO: 6 - DNA, 20 bp, synthetic construct
  source 1..20: mol_type = other DNA
ctgggtcacgttggatgagg

SEQ ID NO: 7 - DNA, 20 bp, synthetic construct
  source 1..20: mol_type = other DNA
aggtccctgtcatgcttctg

SEQ ID NO: 8 - DNA, 20 bp, synthetic construct
  source 1..20: mol_type = other DNA
tctggacccattccttcttg

SEQ ID NO: 9 - DNA, 20 bp, synthetic construct
  source 1..20: mol_type = other DNA
ttgtgcgaaaagaagtgcag

SEQ ID NO: 10 - DNA, 20 bp, synthetic construct
  source 1..20: mol_type = other DNA
tacaaacacagcctcccaca

SEQ ID NO: 11 - DNA, 21 bp, synthetic construct
  source 1..21: mol_type = other DNA
ggaagcacggcagcagaataa

SEQ ID NO: 12 - DNA, 21 bp, synthetic construct
  source 1..21: mol_type = other DNA
cttgagggagaagtaggaatg

SEQ ID NO: 13 - DNA, 22 bp, synthetic construct
  source 1..22: mol_type = other DNA
gaaatgccaccttttgacagtg

SEQ ID NO: 14 - DNA, 21 bp, synthetic construct
  source 1..21: mol_type = other DNA
ctggatgctctcatcaggaca

SEQ ID NO: 15 - DNA, 24 bp, synthetic construct
  source 1..24: mol_type = other DNA
tttgcttccatgctaatgcgaaag

SEQ ID NO: 16 - DNA, 25 bp, synthetic construct
  source 1..25: mol_type = other DNA
gctctgttgaggtctaaaggctccg

SEQ ID NO: 17 - DNA, 19 bp, synthetic construct
  source 1..19: mol_type = other DNA
cccatccccaggagtcttg

SEQ ID NO: 18 - DNA, 20 bp, synthetic construct
  source 1..20: mol_type = other DNA
ccatgactaggggcactgta

SEQ ID NO: 19 - DNA, 21 bp, synthetic construct
  source 1..21: mol_type = other DNA
gaaggcagagttcagggtctt

SEQ ID NO: 20 - DNA, 21 bp, synthetic construct
  source 1..21: mol_type = other DNA
ggttcctgtctttgtggtgaa

SEQ ID NO: 21 - DNA, 20 bp, synthetic construct
  source 1..20: mol_type = other DNA
tcatttccgataaggcttgg

SEQ ID NO: 22 - DNA, 20 bp, synthetic construct
  source 1..20: mol_type = other DNA
ataactgcacccacttccca

SEQ ID NO: 23 - DNA, 20 bp, synthetic construct
  source 1..20: mol_type = other DNA
gccaccacgctcttctgcct

SEQ ID NO: 24 - DNA, 20 bp, synthetic construct
  source 1..20: mol_type = other DNA
ggctgatggtgtgggtgagg

SEQ ID NO: 25 - DNA, 21 bp, synthetic construct
  source 1..21: mol_type = other DNA
tctaaagtcgatccgcgacat

SEQ ID NO: 26 - DNA, 21 bp, synthetic construct
  source 1..21: mol_type = other DNA
ctacgggcagtggtgaaaact

SEQ ID NO: 27 - DNA, 20 bp, synthetic construct
  source 1..20: mol_type = other DNA
tgctgcataatcagctacgg

SEQ ID NO: 28 - DNA, 20 bp, synthetic construct
  source 1..20: mol_type = other DNA
gctggtcacattgagaagca

SEQ ID NO: 29 - DNA, 20 bp, synthetic construct
  source 1..20: mol_type = other DNA
ctacagcaacagggtggtgg

SEQ ID NO: 30 - DNA, 18 bp, synthetic construct
  source 1..18: mol_type = other DNA
tatgggggtctgggatgg